European Patent Specification EP 4 049 535 B1, published November 27, 2024. Title: GENETICALLY MODIFIED MICE AND ENGRAFTMENT. Applicant: REGENERON PHARMACEUTICALS, INC. YALE UNIVERSITY INSTITUTE FOR RESEARCH IN BIOMEDICINE (IRB). Application EP. The sequence listing filed with the application follows.

SEQUENCE LISTING (12 sequences)

SEQ ID NO: 1 - DNA, 18 bp, Artificial Sequence
  Synthetic primer
ccaccacccatggatctc

SEQ ID NO: 2 - DNA, 21 bp, Artificial Sequence
  Synthetic primer
aaagcagaacatctggagcag

SEQ ID NO: 3 - DNA, 20 bp, Artificial Sequence
  Synthetic primer
caggactgaaaagggaatca

SEQ ID NO: 4 - DNA, 20 bp, Artificial Sequence
  Synthetic primer
cgttggaaggccttgaattt

SEQ ID NO: 5 - DNA, 20 bp, Artificial Sequence
  Synthetic primer
gtacgctgtgaaggcatcaa

SEQ ID NO: 6 - DNA, 20 bp, Artificial Sequence
  Synthetic primer
atcccatccaacaccttgag

SEQ ID NO: 7 - DNA, 21 bp, Artificial Sequence
  Synthetic primer
ccagtccaaaaatgaggaagc

SEQ ID NO: 8 - DNA, 20 bp, Artificial Sequence
  Synthetic primer
cagcgttttcagagggctat

SEQ ID NO: 9 - DNA, 20 bp, Artificial Sequence
  Synthetic primer
ggcgtctcctgaacctgagt

SEQ ID NO: 10 - DNA, 20 bp, Artificial Sequence
  Synthetic primer
ggggatgacaagcagaaagt

SEQ ID NO: 11 - DNA, 20 bp, Artificial Sequence
  Synthetic primer
gtacgctgtgaaggcatcaa

SEQ ID NO: 12 - DNA, 20 bp, Artificial Sequence
  Synthetic primer
atcccatccaacaccttgag